European Patent Application EP 4 130 727 A1, published February 8, 2023. Title: Ligand-target interaction analysis by photochemically induced dynamic nuclear polarization (photo-CIDNP) enhanced NMR spectroscopy. Applicant: ETH Zurich. The sequence listing filed with the application follows.

SEQUENCE LISTING (4 sequences)

SEQ ID NO: 1 - protein, 5 aa, Artificial Sequence
  Peptide 1
WVSAV

SEQ ID NO: 2 - protein, 9 aa, Artificial Sequence
  Peptide 2
  MOD_RES (9)..(9): AMIDATION
WENEQVSAV

SEQ ID NO: 3 - protein, 5 aa, Artificial Sequence
  Peptide 3
WEQLT

SEQ ID NO: 4 - protein, 5 aa, Artificial Sequence
  Peptide 4
  MOD_RES (5)..(5): AMIDATION
WVSAV